European Patent Specification EP 3 697 404 B1, published March 26, 2025. Title: Compositions and Methods for Broad-Spectrum Antiviral Therapy. Applicant: Avalon Flaviviral (HK) Limited. The sequence listing filed with the application follows.

SEQUENCE LISTING (1 sequence)

SEQ ID NO: 1 - protein, 80 aa, Homo sapiens
GEKRTAHNAIEKRYRSSINDKIIELKDLVVGTEAKLNKSAVLRKAIDYIRFLQHSNQKLKQENLSLRTAVHKSKSLKDLV